European Patent Specification EP 3 539 037 B1, published June 14, 2023. Title: METHODE DE PREDICTION DE LA RECONNAISSANCE CROISEE DE CIBLES PAR DES ANTICORPS DIFFERENTS. Applicant: INSTITUT NATIONAL DE RECHERCHE AGRONOMIQUE et al. The sequence listing filed with the application follows.

SEQUENCE LISTING (45 sequences)

SEQ ID NO: 1 - protein, 26 aa, artificial sequence
  FR1
MEVQLQESGGGLVQAGASLKLSCAAS

SEQ ID NO: 2 - protein, 26 aa, artificial sequence
  FR1
MEVQLVQSGAEVKKPGASVKVSCKAS

SEQ ID NO: 3 - protein, 17 aa, artificial sequence
  FR2
MGWFRQAPGKEREFVAA

SEQ ID NO: 4 - protein, 18 aa, artificial sequence
  FR2
HINWVRQAPGQGLEWMGW

SEQ ID NO: 5 - protein, 39 aa, artificial sequence
  FR3
TKYADSVKGRFAISRDNDKNTVWLRMNSLKPEDTAVYYC

SEQ ID NO: 6 - protein, 38 aa, artificial sequence
  FR3
NYAQKFQGWVTMTRDTAISTAYMEVNGLKSDDTAVYYC

SEQ ID NO: 7 - protein, 11 aa, artificial sequence
  FR4
WGQGTQVTVSS

SEQ ID NO: 8 - protein, 128 aa, artificial sequence
  4N1H
MEVQLQESGGGLVQAGASLKLSCAASGRTFSSYAMGWFRQAPGKEREFVAAISRSGGDTKYADSVKGRFAISRDNDKNTVWLRMNSLKPEDTAVYYCAATTYASLSDTYIGEHIYDDWGQGTQVTVSS

SEQ ID NO: 9 - protein, 139 aa, artificial sequence
  4N1H - tag myc
MEVQLQESGGGLVQAGASLKLSCAASGRTFSSYAMGWFRQAPGKEREFVAAISRSGGDTKYADSVKGRFAISRDNDKNTVWLRMNSLKPEDTAVYYCAATTYASLSDTYIGEHIYDDWGQGTQVTVSSEQKLISEEDLE

SEQ ID NO: 10 - protein, 145 aa, artificial sequence
  4N1H - tag his
MEVQLQESGGGLVQAGASLKLSCAASGRTFSSYAMGWFRQAPGKEREFVAAISRSGGDTKYADSVKGRFAISRDNDKNTVWLRMNSLKPEDTAVYYCAATTYASLSDTYIGEHIYDDWGQGTQVTVSSEQKLISEEDLEHHHHHH

SEQ ID NO: 11 - protein, 127 aa, artificial sequence
  3SM5
MEVQLVQSGAEVKKPGASVKVSCKASGYTFTDYHINWVRQAPGQGLEWMGWIHPNSGDTNYAQKFQGWVTMTRDTAISTAYMEVNGLKSDDTAVYYCARGGLEPRSVDYYYYGMDVWGQGTTVTVSS

SEQ ID NO: 12 - protein, 138 aa, artificial sequence
  3SM5 - tag myc
MEVQLVQSGAEVKKPGASVKVSCKASGYTFTDYHINWVRQAPGQGLEWMGWIHPNSGDTNYAQKFQGWVTMTRDTAISTAYMEVNGLKSDDTAVYYCARGGLEPRSVDYYYYGMDVWGQGTTVTVSSEQKLISEEDLE

SEQ ID NO: 13 - protein, 144 aa, artificial sequence
  3SM5 - tag his
MEVQLVQSGAEVKKPGASVKVSCKASGYTFTDYHINWVRQAPGQGLEWMGWIHPNSGDTNYAQKFQGWVTMTRDTAISTAYMEVNGLKSDDTAVYYCARGGLEPRSVDYYYYGMDVWGQGTTVTVSSEQKLISEEDLEHHHHHH

SEQ ID NO: 14 - protein, 8 aa, artificial sequence
  CDR1 238D2
GFTFSSYA

SEQ ID NO: 15 - protein, 8 aa, artificial sequence
  CDR2 238D2
IKSSGDST

SEQ ID NO: 16 - protein, 15 aa, artificial sequence
  CDR3 238D2
AKSRVSRTGLYTYDN

SEQ ID NO: 17 - protein, 8 aa, artificial sequence
  CDR1 238D4
GRTFNNYA

SEQ ID NO: 18 - protein, 12 aa, artificial sequence
  CDR2 238D4
ITRSGVRSGVSA

SEQ ID NO: 19 - protein, 17 aa, artificial sequence
  CDR3 238D4
AASAIGSGALRRFEYDY

SEQ ID NO: 20 - protein, 7 aa, artificial sequence
  CDR1 4N1H
GRTFSSY

SEQ ID NO: 21 - protein, 6 aa, artificial sequence
  CDR2 4N1H
SRSGGD

SEQ ID NO: 22 - protein, 18 aa, artificial sequence
  CDR3 4N1H
TTYASLSDTYIGEHIYDD

SEQ ID NO: 23 - protein, 7 aa, artificial sequence
  CDR1 3SM5
GYTFTDY

SEQ ID NO: 24 - protein, 6 aa, artificial sequence
  CDR2 3SM5
HPNSGD

SEQ ID NO: 25 - protein, 17 aa, artificial sequence
  CDR3 3SM5
GGLEPRSVDYYYYGMDV

SEQ ID NO: 26 - protein, 8 aa, artificial sequence
  CDR1 238D2 simplifié
  MISC_FEATURE (1)..(1): Xaa = A, G, S, T, C or P
  MISC_FEATURE (2)..(2): Xaa = Y, F or W
  MISC_FEATURE (3)..(3): Xaa = A, G, S, T, C or P
  MISC_FEATURE (4)..(4): Xaa = Y, F or W
  MISC_FEATURE (5)..(6): Xaa = A, G, S, T, C or P
  MISC_FEATURE (7)..(7): Xaa = Y, F or W
  MISC_FEATURE (8)..(8): Xaa = A, G, S, T, C or P
XXXXXXXX

SEQ ID NO: 27 - protein, 8 aa, artificial sequence
  CDR2 238D2 simplifié
  MISC_FEATURE (1)..(1): Xaa = I, L, F, M or V
  MISC_FEATURE (2)..(2): Xaa = H, K or R
  MISC_FEATURE (3)..(5): Xaa = A, G, S, T, C or P
  MISC_FEATURE (6)..(6): Xaa = D or E
  MISC_FEATURE (7)..(8): Xaa = A, G, S, T, C or P
XXXXXXXX

SEQ ID NO: 28 - protein, 15 aa, artificial sequence
  CDR3 238D2 simplifié
  MISC_FEATURE (1)..(1): Xaa = A, G, S, T, C or P
  MISC_FEATURE (2)..(2): Xaa = H, K or R
  MISC_FEATURE (3)..(3): Xaa = A, G, S, T, C or P
  MISC_FEATURE (4)..(4): Xaa = H, K or R
  MISC_FEATURE (5)..(5): Xaa = I, L, F, M or V
  MISC_FEATURE (6)..(6): Xaa = A, G, S, T, C or P
  MISC_FEATURE (6)..(6): Xaa = H, K or R
  misc_feature (7)..(7): Xaa can be any naturally occurring amino acid
  MISC_FEATURE (8)..(9): Xaa = A, G, S, T, C or P
  MISC_FEATURE (10)..(10): Xaa = I, L, F, M or V
  MISC_FEATURE (11)..(11): Xaa = Y, F or W
  MISC_FEATURE (12)..(12): Xaa = A, G, S, T, C or P
  MISC_FEATURE (13)..(13): Xaa = Y, F or W
  MISC_FEATURE (14)..(14): Xaa = D or E
  MISC_FEATURE (15)..(15): Xaa = N or Q
XXXXXXXXXXXXXXX

SEQ ID NO: 29 - protein, 8 aa, artificial sequence
  CDR1 238D4 simplifié
  MISC_FEATURE (1)..(1): Xaa = A, G, S, T, C or P
  MISC_FEATURE (2)..(2): Xaa = H, K or R
  MISC_FEATURE (3)..(3): Xaa = A, G, S, T, C or P
  MISC_FEATURE (4)..(4): Xaa = Y, F or W
  MISC_FEATURE (5)..(6): Xaa = N or Q
  MISC_FEATURE (7)..(7): Xaa = Y, F or W
  MISC_FEATURE (8)..(8): Xaa = A, G, S, T, C or P
XXXXXXXX

SEQ ID NO: 30 - protein, 12 aa, artificial sequence
  CDR2 238D4 simplifié
  MISC_FEATURE (1)..(1): Xaa = I, L, F, M or V
  MISC_FEATURE (2)..(2): Xaa = A, G, S, T, C or P
  MISC_FEATURE (3)..(3): Xaa = H, K or R
  MISC_FEATURE (4)..(5): Xaa = A, G, S, T, C or P
  MISC_FEATURE (6)..(6): Xaa = I, L, F, M or V
  MISC_FEATURE (7)..(7): Xaa = H, K or R
  MISC_FEATURE (8)..(9): Xaa = A, G, S, T, C or P
  MISC_FEATURE (10)..(10): Xaa = I, L, F, M or V
  MISC_FEATURE (11)..(12): Xaa = A, G, S, T, C or P
XXXXXXXXXXXX

SEQ ID NO: 31 - protein, 17 aa, artificial sequence
  CDR3 238D4 simplifié
  MISC_FEATURE (1)..(4): Xaa = A, G, S, T, C or P
  MISC_FEATURE (5)..(5): Xaa = I, L, F, M or V
  MISC_FEATURE (6)..(9): Xaa = A, G, S, T, C or P
  MISC_FEATURE (10)..(10): Xaa = I, L, F, M or V
  MISC_FEATURE (11)..(12): Xaa = H, K or R
  MISC_FEATURE (13)..(13): Xaa = Y, F or W
  MISC_FEATURE (14)..(14): Xaa = D or E
  MISC_FEATURE (15)..(15): Xaa = Y, F or W
  MISC_FEATURE (16)..(16): Xaa = D or E
  MISC_FEATURE (17)..(17): Xaa = Y, F or W
XXXXXXXXXXXXXXXXX

SEQ ID NO: 32 - protein, 7 aa, artificial sequence
  CDR1 4N1H simplifié
  MISC_FEATURE (1)..(1): Xaa = A, G, S, T, C or P
  MISC_FEATURE (2)..(2): Xaa = H, K or R
  MISC_FEATURE (3)..(3): Xaa = A, G, S, T, C or P
  MISC_FEATURE (4)..(4): Xaa = Y, F or W
  MISC_FEATURE (5)..(6): Xaa = A, G, S, T, C or P
  MISC_FEATURE (7)..(7): Xaa = Y, F or W
XXXXXXX

SEQ ID NO: 33 - protein, 6 aa, artificial sequence
  CDR2 4N1H simplifié
  MISC_FEATURE (1)..(1): Xaa = A, G, S, T, C or P
  MISC_FEATURE (2)..(2): Xaa = H, K or R
  MISC_FEATURE (3)..(5): Xaa = A, G, S, T, C or P
  MISC_FEATURE (6)..(6): Xaa = D or E
XXXXXX

SEQ ID NO: 34 - protein, 18 aa, artificial sequence
  CDR3 4N1H simplifié
  MISC_FEATURE (1)..(2): Xaa = A, G, S, T, C or P
  MISC_FEATURE (3)..(3): Xaa = Y, F or W
  MISC_FEATURE (4)..(5): Xaa = A, G, S, T, C or P
  MISC_FEATURE (6)..(6): Xaa = I, L, F, M or V
  MISC_FEATURE (7)..(7): Xaa = A, G, S, T, C or P
  MISC_FEATURE (8)..(8): Xaa = D or E
  MISC_FEATURE (9)..(9): Xaa = A, G, S, T, C or P
  MISC_FEATURE (10)..(10): Xaa = Y, F or W
  MISC_FEATURE (11)..(11): Xaa = I, L, F, M or V
  MISC_FEATURE (12)..(12): Xaa = A, G, S, T, C or P
  MISC_FEATURE (13)..(13): Xaa = D or E
  MISC_FEATURE (14)..(14): Xaa = H, K or R
  MISC_FEATURE (15)..(15): Xaa = I, L, F, M or V
  MISC_FEATURE (16)..(16): Xaa = Y, F or W
  MISC_FEATURE (17)..(18): Xaa = D or E
XXXXXXXXXXXXXXXXXX

SEQ ID NO: 35 - protein, 7 aa, artificial sequence
  CDR1 3SM5 simplifié
  MISC_FEATURE (1)..(1): Xaa = A, G, S, T, C or P
  MISC_FEATURE (2)..(2): Xaa = Y, F or W
  MISC_FEATURE (3)..(3): Xaa = A, G, S, T, C or P
  MISC_FEATURE (4)..(4): Xaa = Y, F or W
  MISC_FEATURE (5)..(5): Xaa = A, G, S, T, C or P
  MISC_FEATURE (6)..(6): Xaa = D or E
  MISC_FEATURE (7)..(7): Xaa = Y, F or W
XXXXXXX

SEQ ID NO: 36 - protein, 6 aa, artificial sequence
  CDR2 3SM5 simplifié
  MISC_FEATURE (1)..(1): Xaa = H, K or R
  MISC_FEATURE (2)..(2): Xaa = A, G, S, T, C or P
  MISC_FEATURE (3)..(3): Xaa = N or Q
  MISC_FEATURE (4)..(5): Xaa = A, G, S, T, C or P
  misc_feature (6)..(6): Xaa can be any naturally occurring amino acid
  MISC_FEATURE (7)..(7): Xaa = D or E
XXXXXX

SEQ ID NO: 37 - protein, 17 aa, artificial sequence
  CDR3 3SM5 simplifié
  MISC_FEATURE (1)..(2): Xaa = A, G, S, T, C or P
  MISC_FEATURE (3)..(3): Xaa = I, L, F, M or V
  MISC_FEATURE (4)..(4): Xaa = D or E
  MISC_FEATURE (5)..(5): Xaa = A, G, S, T, C or P
  MISC_FEATURE (6)..(6): Xaa = H, K or R
  MISC_FEATURE (7)..(7): Xaa = A, G, S, T, C or P
  MISC_FEATURE (8)..(8): Xaa = I, L, F, M or V
  MISC_FEATURE (9)..(9): Xaa = D or E
  MISC_FEATURE (10)..(13): Xaa = Y, F or W
  MISC_FEATURE (14)..(14): Xaa = A, G, S, T, C or P
  MISC_FEATURE (15)..(15): Xaa = I, L, F, M or V
  MISC_FEATURE (16)..(16): Xaa = D or E
  MISC_FEATURE (17)..(17): Xaa = I, L, F, M or V
XXXXXXXXXXXXXXXXX

SEQ ID NO: 38 - protein, 177 aa, artificial sequence
  AviTag - 3SM5 - tag myc
MGSSHHHHHHSSGLVPRGSHMSGLNDIFEAQKIEWHEDPNSEVQLVQSGAEVKKPGASVKVSCKASGYTFTDYHINWVRQAPGQGLEWMGWIHPNSGDTNYAQKFQGWVTMTRDTAISTAYMEVNGLKSDDTAVYYCARGGLEPRSVDYYYYGMDVWGQGTTVTVSSEQKLISEEDL

SEQ ID NO: 39 - protein, 134 aa, artificial sequence
  238D2- tag myc
MEVQLVESGGGLVQTGGSLRLSCAASGFTFSSYAMSWVRQAPGKGLEWVSGIKSSGDSTRYAGSVKGRFTISRDNAKNMLYLQMYSLKPEDTAVYYCAKSRVSRTGLYTYDNRGQGTQVTVSSEQKLISEEDLE

SEQ ID NO: 40 - protein, 140 aa, artificial sequence
  238D2- tag his
MEVQLVESGGGLVQTGGSLRLSCAASGFTFSSYAMSWVRQAPGKGLEWVSGIKSSGDSTRYAGSVKGRFTISRDNAKNMLYLQMYSLKPEDTAVYYCAKSRVSRTGLYTYDNRGQGTQVTVSSEQKLISEEDLEHHHHHH

SEQ ID NO: 41 - protein, 173 aa, artificial sequence
  AviTag - 238D2 - tag myc
MGSSHHHHHHSSGLVPRGSHMSGLNDIFEAQKIEWHEDPNSEVQLVESGGGLVQTGGSLRLSCAASGFTFSSYAMSWVRQAPGKGLEWVSGIKSSGDSTRYAGSVKGRFTISRDNAKNMLYLQMYSLKPEDTAVYYCAKSRVSRTGLYTYDNRGQGTQVTVSSEQKLISEEDL

SEQ ID NO: 42 - protein, 140 aa, artificial sequence
  238D4- tag myc
MEVQLMESGGGLVQAGGSLRLSCAASGRTFNNYAMGWFRRAPGKEREFVAAITRSGVRSGVSAIYGDSVKDRFTISRDNAKNTLYLQMNSLKPEDTAVYTCAASAIGSGALRRFEYDYSGQGTQVTVSSEQKLISEEDLE

SEQ ID NO: 43 - protein, 146 aa, artificial sequence
  238D4- tag his
MEVQLMESGGGLVQAGGSLRLSCAASGRTFNNYAMGWFRRAPGKEREFVAAITRSGVRSGVSAIYGDSVKDRFTISRDNAKNTLYLQMNSLKPEDTAVYTCAASAIGSGALRRFEYDYSGQGTQVTVSSEQKLISEEDLEHHHHHH

SEQ ID NO: 44 - protein, 182 aa, artificial sequence
  Ovalbumine - tag his
MGSSHHHHHHSSGLVPRGSHMASMTGGQQMGRGSEFELRRQACGRTRAPPPPPLRSGCEVQLQESGGSGQAGGSLRLSCAASGDTVRTMAWFRQAPGQEREGVAGFNLPISRPYYADGMKARFTISGDKSKNTVTLQMDNLAPEDTANYYCAATRYTLDLSSRIFQGDFDHWGHGTQVTVSS

SEQ ID NO: 45 - protein, 498 aa, Homo sapiens
MEGISIYTSDNYTEEMGSGDYDSMKEPCFREENANFNKIFLPTIYSIIFLTGIVGNGLVILVMGYQKKLRSMTDKYRLHLSVADLLFVITLPFWAVDAVANWYFGNFLCKAVHVIYTVNLYSSVWILAFISLDRYLAIVHATNSQRPRKLLAEKVVYVGVWIPALLLTIPDFIFANVSEADDRYICDRFYPNDLWVVVFQFQHIMVGLILPGIVILSCYCIIISKLSHSGSNIFEMLRIDEGLRLKIYKDTEGYYTIGIGHLLTKSPSLNAAKSELDKAIGRNTNGVITKDEAEKLFNQDVDAAVRGILRNAKLKPVYDSLDAVRRAALINMVFQMGETGVAGFTNSLRMLQQKRWDEAAVNLAKSRWYNQTPNRAKRVITTFRTGTWDAYGSKGHQKRKALKTTVILILAFFACWLPYYIGISIDSFILLEIIKQGCEFENTVHKWISITEALAFFHCCLNPILYAFLGAKFKTSAQHALTSVSRGSSGRPLEVLFQ